European Patent Specification EP 4 243 873 B1, published February 19, 2025. Title: THERAPEUTIC-OLIGONUCLEOTIDES ACTIVATED BY NUCLEASES. Applicant: HERNANDEZ Frank J. The sequence listing filed with the application follows.

SEQUENCE LISTING (5 sequences)

SEQ ID NO: 1 - RNA, 11 nt, Artificial Sequence
  TT probe with FAM and RQ
  misc_feature 1,3,7,11: /note="c = 2’-O-Methyl Cytosine"
  misc_feature 2,9,10: /note="u = um"
  misc_feature 4,8: /note="g= 2’-O-Methyl Guanine"
  misc_feature 5,6: /note="t = deoxythymidine"
cucgttcguuc

SEQ ID NO: 2 - RNA, 10 nt, Artificial Sequence
  TTprobe2
  misc_feature 1,2,3,4,7,8,9,10: /note="u = um"
  misc_feature 5,6: /note="t = deoxythymidine"
uuuuttuuuu

SEQ ID NO: 3 - RNA, 11 nt, Artificial Sequence
  Upstream GeTT
  misc_feature 1,2,3,4,8,9,10,11: /note="u = um"
  misc_feature 5: /note="n = Ge nucleoside analogue"
  misc_feature 6,7: /note="t =deoxythymidine"
uuuunttuuuu

SEQ ID NO: 4 - RNA, 11 nt, Artificial Sequence
  Downstream TTGe
  misc_feature 1,2,3,4,8,9,10,11: /note="u = um"
  misc_feature 5,6: /note="t = deoxythimidine"
  misc_feature 7: /note="n = Ge nucleoside analogue"
uuuuttnuuuu

SEQ ID NO: 5 - RNA, 10 nt, Artificial Sequence
  TT probe original
  misc_feature 1,3,7,10: /note="C =2’-O-Methyl Cytosine"
  misc_feature 2,9: /note="u = um"
  misc_feature 4,8: /note="g = 2’-O-Methyl Guanine"
  misc_feature 5,6: /note="t = Deoxythymidine"
cucgttcguc